European Patent Application EP 4 707 381 A1, published March 11, 2026. Title: NITROGEN-FIXING BACTERIUM, AND METHOD FOR PRODUCING AMMONIA-, AMINO ACID- OR PROTEIN-CONTAINING CULTURE USING NITROGEN-FIXING 5 BACTERIUM. Applicant: Kikkoman Corporation. Application EP 24797228.4, filed April 26, 2024. The sequence listing filed with the application follows.

SEQUENCE LISTING (32 sequences)

SEQ ID NO: 1 - DNA, 34 bp, synthetic construct
  source 1..34: mol_type = other DNA
gacgagttcttctgaaaggatctaggtgaagatc

SEQ ID NO: 2 - DNA, 34 bp, synthetic construct
  source 1..34: mol_type = other DNA
agccttcgcgcatgctgtttcctgtgtgaaattg

SEQ ID NO: 3 - DNA, 31 bp, synthetic construct
  source 1..31: mol_type = other DNA
aggaaacagcatgcgcgaaggctgccggatc

SEQ ID NO: 4 - DNA, 33 bp, synthetic construct
  source 1..33: mol_type = other DNA
agtgagggttaatttcagttcaggcgcacgaag

SEQ ID NO: 5 - DNA, 34 bp, synthetic construct
  source 1..34: mol_type = other DNA
cgtgcgcctgaactgaaattaaccctcactaaag

SEQ ID NO: 6 - DNA, 33 bp, synthetic construct
  source 1..33: mol_type = other DNA
ttcacctagatcctttcagaagaactcgtcaag

SEQ ID NO: 7 - DNA, 20 bp, synthetic construct
  source 1..20: mol_type = other DNA
aaggatctaggtgaagatcc

SEQ ID NO: 8 - DNA, 19 bp, synthetic construct
  source 1..19: mol_type = other DNA
tcagttcaggcgcacgaag

SEQ ID NO: 9 - DNA, 33 bp, synthetic construct
  source 1..33: mol_type = other DNA
gtgcgcctgaactgatcagaagaactcgtcaag

SEQ ID NO: 10 - DNA, 33 bp, synthetic construct
  source 1..33: mol_type = other DNA
ttcacctagatccttctaccgggtaggggaggc

SEQ ID NO: 11 - DNA, 25 bp, synthetic construct
  source 1..25: mol_type = other DNA
taatcatcggctcgtataatgtgtg

SEQ ID NO: 12 - DNA, 34 bp, synthetic construct
  source 1..34: mol_type = other DNA
acgagccgatgattaattgtcaacagctcatttc

SEQ ID NO: 13 - DNA, 25 bp, synthetic construct
  source 1..25: mol_type = other DNA
atggtgcacgtagacaccgactatc

SEQ ID NO: 14 - DNA, 25 bp, synthetic construct
  source 1..25: mol_type = other DNA
agagttcggactcgagcagggtttc

SEQ ID NO: 15 - DNA, 19 bp, synthetic construct
  source 1..19: mol_type = other DNA
gcttatcgatgataagctg

SEQ ID NO: 16 - DNA, 22 bp, synthetic construct
  source 1..22: mol_type = other DNA
agctgtttcctgtgtgaaattg

SEQ ID NO: 17 - DNA, 34 bp, synthetic construct
  source 1..34: mol_type = other DNA
ttatcatcgataagctcgcgggtgaaaggaacac

SEQ ID NO: 18 - DNA, 34 bp, synthetic construct
  source 1..34: mol_type = other DNA
acacaggaaacagctccttggaagaaggctcctg

SEQ ID NO: 19 - DNA, 21 bp, synthetic construct
  source 1..21: mol_type = other DNA
ccttcatcaaagcctatcgtg

SEQ ID NO: 20 - DNA, 22 bp, synthetic construct
  source 1..22: mol_type = other DNA
tcagatcttgcgcatgtggatg

SEQ ID NO: 21 - DNA, 34 bp, synthetic construct
  source 1..34: mol_type = other DNA
tgcgggaggtggatcaattaaccctcactaaagg

SEQ ID NO: 22 - DNA, 34 bp, synthetic construct
  source 1..34: mol_type = other DNA
acagcttgtctgtaagtcagaagaactcgtcaag

SEQ ID NO: 23 - DNA, 34 bp, synthetic construct
  source 1..34: mol_type = other DNA
gacgagttcttctgacttacagacaagctgtgac

SEQ ID NO: 24 - DNA, 35 bp, synthetic construct
  source 1..35: mol_type = other DNA
aggctttgatgaaggtcactgcccgctttccagtc

SEQ ID NO: 25 - DNA, 18 bp, synthetic construct
  source 1..18: mol_type = other DNA
aattaaccctcactaaag

SEQ ID NO: 26 - DNA, 22 bp, synthetic construct
  source 1..22: mol_type = other DNA
tcagatcttgcgcatgtggatg

SEQ ID NO: 27 - DNA, 34 bp, synthetic construct
  source 1..34: mol_type = other DNA
tgcgggaggtggatcgtttgacagcttatcatcg

SEQ ID NO: 28 - DNA, 33 bp, synthetic construct
  source 1..33: mol_type = other DNA
ccggcagccttcgcgcatgctgtttcctgtgtg

SEQ ID NO: 29 - DNA, 34 bp, synthetic construct
  source 1..34: mol_type = other DNA
acaggaaacagcatgcgcgaaggctgccggatcg

SEQ ID NO: 30 - DNA, 37 bp, synthetic construct
  source 1..37: mol_type = other DNA
tagtgagggttaatttcagatcttgcgcatgtggatg

SEQ ID NO: 31 - DNA, 23 bp, synthetic construct
  source 1..23: mol_type = other DNA
ggcgagtagagtcttgaagatgg

SEQ ID NO: 32 - DNA, 24 bp, synthetic construct
  source 1..24: mol_type = other DNA
tgttgacgaagataggtgggaagc